European Patent Specification EP 3 920 954 B9, published October 4, 2023. Title: ANTIMICROBIAL PEPTIDE FOR ONYCHOMYCOSIS. Applicant: CBMR Scientific Nanoscience B.V. The sequence listing filed with the application follows.

SEQUENCE LISTING (5 sequences)

SEQ ID NO: 1 - protein, 10 aa, Homo sapiens
RRRRSVQWCA

SEQ ID NO: 2 - protein, 10 aa, Artificial Sequence
  Reverse hLF2-11
ACWQVSRRRR

SEQ ID NO: 3 - protein, 11 aa, Homo sapiens
GRRRRSVQWCA

SEQ ID NO: 4 - protein, 11 aa, Artificial Sequence
  Reverse hLF1-11
ACWQVSRRRRG

SEQ ID NO: 5 - protein, 12 aa, Artificial Sequence
  cysteine - hLF1-11
CGRRRRSVQWCA